European Patent Specification EP 3 425 054 B1, published December 20, 2023. Title: Mutant cytochrome protein and use thereof. Applicant: Arkray, Inc. Ultizyme International Ltd. The sequence listing filed with the application follows.

SEQUENCE LISTING (19 sequences)

SEQ ID NO: 1 - DNA, 3706 bp, Burkholderia cepacia
  CDS (258)..(761)
  CDS (764)..(2380)
  CDS (2386)..(3660)
aagctttctgtttgattgcacgcgattctaaccgagcgtctgtgaggcggaacgcgacatgcttcgtgtcgcacacgtgtcgcgccgacgacacaaaaatgcagcgaaatggctgatcgttacgaatggctgacacattgaatggactataaaaccattgtccgttccggaatgtgcgcgtacatttcaggtccgcgccgatttttgagaaatatcaagcgtggttttcccgaatccggtgttcgagagaaggaaacatgcacaacgacaacactccccactcgcgtcgccacggcgacgcagccgcatcaggcatcacgcggcgtcaatggttgcaaggcgcgctggcgctgaccgcagcgggcctcacgggttcgctgacattgcgggcgcttgcagacaaccccggcactgcgccgctcgatacgttcatgacgctttccgaatcgctgaccggcaagaaagggctcagccgcgtgatcggcgagcgcctgctgcaggcgctgcagaagggctcgttcaagacggccgacagcctgccgcagctcgccggcgcgctcgcgtccggttcgctgacgcctgaacaggaatcgctcgcactgacgatcctcgaggcctggtatctcggcatcgtcgacaacgtcgtgattacgtacgaggaagcattaatgttcggcgtcgtgtccgatacgctcgtgatccgttcgtattgccccaacaaacccggcttctgggccgacaaaccgatcgagaggcaagcctgatggccgataccgatacgcaaaaggccgacgtcgtcgtcgttggatcgggtgtcgcgggcgcgatcgtcgcgcatcagctcgcgatggcgggcaaggcggtgatcctgctcgaagcgggcccgcgcatgccgcgctgggaaatcgtcgagcgcttccgcaatcagcccgacaagatggacttcatggcgccgtacccgtcgagcccctgggcgccgcatcccgagtacggcccgccgaacgactacctgatcctgaagggcgagcacaagttcaactcgcagtacatccgcgcggtgggcggcacgacgtggcactgggccgcgtcggcgtggcgcttcattccgaacgacttcaagatgaagagcgtgtacggcgtcggccgcgactggccgatccagtacgacgatctcgagccgtactatcagcgcgcggaggaagagctcggcgtgtggggcccgggccccgaggaagatctgtactcgccgcgcaagcagccgtatccgatgccgccgctgccgttgtcgttcaacgagcagaccatcaagacggcgctgaacaactacgatccgaagttccatgtcgtgaccgagccggtcgcgcgcaacagccgcccgtacgacggccgcccgacttgttgcggcaacaacaactgcatgccgatctgcccgatcggcgcgatgtacaacggcatcgtgcacgtcgagaaggccgaacgcgccggcgcgaagctgatcgagaacgcggtcgtctacaagctcgagacgggcccggacaagcgcatcgtcgcggcgctctacaaggacaagacgggcgccgagcatcgcgtcgaaggcaagtatttcgtgctcgccgcgaacggcatcgagacgccgaagatcctgctgatgtccgcgaaccgcgatttcccgaacggtgtcgcgaacagctcggacatggtcggccgcaacctgatggaccatccgggcaccggcgtgtcgttctatgcgagcgagaagctgtggccgggccgcggcccgcaggagatgacgtcgctgatcggtttccgcgacggtccgttccgcgcgaccgaagcggcgaagaagatccacctgtcgaacctgtcgcgcatcgaccaggagacgcagaagatcttcaaggccggcaagctgatgaagcccgacgagctcgacgcgcagatccgcgaccgttccgcacgctacgtgcagttcgactgcttccacgaaatcctgccgcaacccgagaaccgcatcgtgccgagcaagacggcgaccgatgcgatcggcattccgcgccccgagatcacgtatgcgatcgacgactacgtgaagcgcggcgccgcgcatacgcgcgaggtctacgcgaccgccgcgaaggtgctcggcggcacggacgtcgtgttcaacgacgaattcgcgccgaacaatcacatcacgggctcgacgatcatgggcgccgatgcgcgcgactccgtcgtcgacaaggactgccgcacgttcgaccatccgaacctgttcatttcgagcagcgcgacgatgccgaccgtcggtaccgtaaacgtgacgctgacgatcgccgcgctcgcgctgcggatgtcggacacgctgaagaaggaagtctgaccgtgcggaaatctactctcactttcctcatcgccggctgcctcgcgttgccgggcttcgcgcgcgcggccgatgcggccgatccggcgctggtcaagcgcggcgaatacctcgcgaccgccggcgactgcatggcctgccacaccgtgaagggcggcaagccgtacgcgggcggccttggcatgccggtaccgatgctcggcaagatctacacgagcaacatcacgcccgatcccgatacgggcatcggcaaatggacgttcgaggacttcgagcgcgcggtgcggcacggcgtgtcgaagaacggcgacaacctgtatccggcgatgccgtacgtgtcgtacgcgaagatcacggacgacgacgtacgcgcgctgtacgcctacttcatgcacggcgtcgagccggtcaagcaggcgccgccgaagaacgagattcccgcgctgctcagcatgcgctggccgctgaagatctggaactggctgttcctgaaggacggcccgtaccagccgaagccgtcgcagagcgccgaatggaatcgcggcgcgtatctggtgcagggtctcgcgcactgcagcacgtgccacacgccgcgcggcatcgcgatgcaggagaagtcgctcgacgaaaccggcggcagcttcctcgcggggtcggtgctcgccggctgggacggctacaacatcacgtcggacccgaatgcggggatcggcagctggacgcagcagcagctcgtgcagtatttgcgcaccggcagcgtgccgggcgtcgcgcaggcggccgggccgatggccgaggcggtcgagcacagcttctcgaagatgaccgaagcggacatcggtgcgatcgccacgtacgtccgcacggtgccggccgttgccgacagcaacgcgaagcagccgcggtcgtcgtggggcaagccggccgaggacgggctgaagctgcgcggtgtcgcgctcgcgtcgtcgggcatcgatccggcgcggctgtatctcggcaactgcgcgacgtgccaccagatgcagggcaagggcacgccggacggctattacccgtcgctgttccacaactccaccgtcggcgcgtcgaatccgtcgaacctcgtgcaggtgatcctgaacggcgtgcagcgcaagatcggcagcgaggatatcgggatgcccgctttccgctacgatctgaacgacgcgcagatcgccgcgctgacgaactacgtgaccgcgcagttcggcaatccggcggcgaaggtgacggagcaggacgtcgcgaagctgcgctgacatagtcgggcgcgccgacacggcgcaaccgataggacaggag

SEQ ID NO: 2 - protein, 168 aa, Burkholderia cepacia
MHNDNTPHSRRHGDAAASGITRRQWLQGALALTAAGLTGSLTLRALADNPGTAPLDTFMTLSESLTGKKGLSRVIGERLLQALQKGSFKTADSLPQLAGALASGSLTPEQESLALTILEAWYLGIVDNVVITYEEALMFGVVSDTLVIRSYCPNKPGFWADKPIERQA

SEQ ID NO: 3 - protein, 539 aa, Burkholderia cepacia
MADTDTQKADVVVVGSGVAGAIVAHQLAMAGKAVILLEAGPRMPRWEIVERFRNQPDKMDFMAPYPSSPWAPHPEYGPPNDYLILKGEHKFNSQYIRAVGGTTWHWAASAWRFIPNDFKMKSVYGVGRDWPIQYDDLEPYYQRAEEELGVWGPGPEEDLYSPRKQPYPMPPLPLSFNEQTIKTALNNYDPKFHVVTEPVARNSRPYDGRPTCCGNNNCMPICPIGAMYNGIVHVEKAERAGAKLIENAVVYKLETGPDKRIVAALYKDKTGAEHRVEGKYFVLAANGIETPKILLMSANRDFPNGVANSSDMVGRNLMDHPGTGVSFYASEKLWPGRGPQEMTSLIGFRDGPFRATEAAKKIHLSNLSRIDQETQKIFKAGKLMKPDELDAQIRDRSARYVQFDCFHEILPQPENRIVPSKTATDAIGIPRPEITYAIDDYVKRGAAHTREVYATAAKVLGGTDVVFNDEFAPNNHITGSTIMGADARDSVVDKDCRTFDHPNLFISSSATMPTVGTVNVTLTIAALALRMSDTLKKEV

SEQ ID NO: 4 - protein, 425 aa, Burkholderia cepacia
MRKSTLTFLIAGCLALPGFARAADAADPALVKRGEYLATAGDCMACHTVKGGKPYAGGLGMPVPMLGKIYTSNITPDPDTGIGKWTFEDFERAVRHGVSKNGDNLYPAMPYVSYAKITDDDVRALYAYFMHGVEPVKQAPPKNEIPALLSMRWPLKIWNWLFLKDGPYQPKPSQSAEWNRGAYLVQGLAHCSTCHTPRGIAMQEKSLDETGGSFLAGSVLAGWDGYNITSDPNAGIGSWTQQQLVQYLRTGSVPGVAQAAGPMAEAVEHSFSKMTEADIGAIATYVRTVPAVADSNAKQPRSSWGKPAEDGLKLRGVALASSGIDPARLYLGNCATCHQMQGKGTPDGYYPSLFHNSTVGASNPSNLVQVILNGVQRKIGSEDIGMPAFRYDLNDAQIAALTNYVTAQFGNPAAKVTEQDVAKLR

SEQ ID NO: 5 - protein, 5 aa, Artificial Sequence
  heme binding site
  misc_feature (2)..(3): Xaa can be any naturally occurring amino acid
CXXCH

SEQ ID NO: 6 - protein, 425 aa, Burkholderia cepacia
MRKSTLTFLLAGCLALPGLARAADSADPAQVKRGEYLAVAGDCMACHTAKGGKPFAGGLGMPVPMLGKIYTSNITPDPDTGIGNWTFEDFERAVRHGVSKNGDNLYPAMPYVSYAKINDDDVQALYAYFMHGVEPVKQAPPKNEIPALLSMRWPLKIWNWLFLKDGVYQPKPEQSAEWNRGAYLVQGLAHCSTCHTPRGIAMQEKSLDETGGSFLSGSVLAGWDGYNITSDPNAGIGGWTQQQLVQYLRTGSVPGLAQAAGPMAEAIEHSFSKMTEADIGAISTYIRTVPAVASGDAKQSRSSWGKPAEDGLKLRGVALASSGIDPARLYLGNCATCHQMQGKGTPDGYYPPLFHNSTVGASNPTNLVQVILNGVQRKAGSEDVGMPAFRHELSDAQIAALTNYLTGQFGNPAAKVTEQDVAKLR

SEQ ID NO: 7 - protein, 428 aa, Burkholderia cenocepacia
MRLPGLSVLVVFFLIATDPASAAGQAADRIAAGKALAVAADCVACHTVQGGQPFAGGLAMPLPMGDIYSTNITPDRQTGIGNYSERDFANVLRKGLRRDGGNLYPAMPYPSYTKFSDDDIANLYAYFMQGVAPVRQPNRAPDFPWPLTMRWPLKIWNALYLREGAYVPKPGRDAEWNRGAYLVQGAAHCGTCHTPRGIGMQELAYDETGVGYLAGAPLAGWQAFNITHDRDAGIGTWTTAQIVQYLRTGNVPGKAQAAGPMAEAVEHSFSRMSERDLNAIAVYLSTVPAAKGADTAPRSTQGRPTDDYVAIRAAAAAGSWTPAGASLYLDHCASCHGMTGAGTTDGFFPSLFANSAVGTATASNLLQVVMHGASVNNGTTHYFMPAFQTELDDDEVVTLVNYLSERFGNGRARVSAAEVAKIRTAPAH

SEQ ID NO: 8 - protein, 425 aa, Burkholderia multivorans
MRKSTLTFLIAGCLALPGLARAADAADPALVKRGEYLATAGDCMACHTVKGGKPYAGGLGMPVPMLGKIYTSNITPDPDTGIGKWTFEDFERAVRHGVSKNGDNLYPAMPYVSYAKITDDDVRALYAYFMHGVEPVKQAPPKNEIPALLSMRWPLKIWNWLFLKDGPYQPKPSQSAEWNRGAYLVQGLAHCSTCHTPRGIAMQEKSLDETGGSFLAGSVLAGWDGYNITSDPNAGIGSWTQQQLVQYLRTGSVPGVAQAAGPMAEAVEHSFSKMTEADIGAIATYVRTVPAVADSNAKQPRSSWGKPAEDGLKLRGVALASSGIDPARLYLGNCATCHQMQGKGTPDGYYPSLFHNSTVGASNPSNLVQVILNGVQRKIGSEDIGMPAFRYDLNDAQIAALTNYLTAQFGNPAAKVTEQDVAKLR

SEQ ID NO: 9 - protein, 425 aa, Burkholderia ubonensis
MLKQTLSFLLAGCLALPGLTRAAEPADAALVKRGEYLAVAGDCMACHTTKGGKPFAGGLGMPVPLLGKIYTSNITPDADTGIGNWSYDDFERAVRRGVSKNGDNLYPAMPYVSYAKVSDDDVKALYAYFMHGVEPVKQTPPKNEIPALLSMRWPLKIWNWLFLKDGAYQPKPSQSVEWNRGAYLVQGLAHCSTCHTPRGIAMQEKSLDETGGSFLSGSLLAGWDGYNITSDQNAGIGGWTQEQLVQYLRTGSVPGVAQAAGPMAEAVEHSFSKMTDADIGAIATYIRTVPAVADSSAKQPRYTWGKPAEDGLRLRGVALASSGIDPARLYLGNCASCHQMQGKGTPDGYYPSLFHNSTVGAPNPSNLVQVILNGVQRKAGSEDVGMPAFRHELSDAQIAALANYLTGQFGNPAAKVTEQDVAKAR

SEQ ID NO: 10 - protein, 425 aa, Burkholderia stagnalis
MLKQSLTFLLAGCLALPGLARAADPADAALVKRGEYLAVAGDCMACHTVKGGKPFAGGLGMPVPMLGKIYTSNITPDADTGIGGWTYDDFERAVRHGVSKNGDNLYPAMPYVSYAKVSDDDVKALYAYFMHGVEPVKQTPPKNEIPALLSMRWPLKIWNWLFLKDGAYQPKPAQSAEWNRGAYLVQGLAHCSTCHTPRGIAMQEKSLDETGGSFLSGSVLAGWDGYNITSDANAGIGGWSQQQLVQYLRTGSVPGVAQAAGPMAEAVEHSFSKMTDADIGAIATYIRTVPAVADSSVKQPRATWGKPAEDGLRLRGVALASSGIDPARLYLGNCASCHQMQGKGTPDGYYPSLFHNSTVGAPNPTNLVQVILNGVQRKAGSEDVGMPAFRHELSDAQIAALANYLTGQFGNPAAKVTEQDVAKLR

SEQ ID NO: 11 - protein, 447 aa, Burkholderia thailandensis
MLKRTLSFVLAGCLALPGLSVAASSAPVAAATSAAAATSASSAPSADAALVERGRYLAVAGDCMACHTAKGGKPFAGGLPMRAPLLGTIYTTNITPDKETGIGDWTFADFERAVRHGVAKNGDNLYPAMPYVSYAKVTDDDVKALYAYFTHGVEPVRQPPRKNDIPWYLSMRWPLKIWNLLFLKEGVYQPKPERSVEWNRGAYLVQGLAHCGTCHTPRAVTLQEKSLDETGGSFLAGSVLSGWDGYNITSDTNAGIGGWSQQQLVQYLRTGSVPGLAQAAGPMAEAVEHSFSQMTDADIGAIATYIRTVPAVADGTAKARSAWGKPAEDGIRLRGVALAATGIDPARLYLGNCASCHQMQGKGTPDGYYPPLLHNSTVGAPNPTNLVQVILNGVARKAGGEDVGMPAFRRELSDAQIAALANYLTAQFGNPAAKVSEQDVAKLRAAQ

SEQ ID NO: 12 - protein, 431 aa, Ralstonia solanacearum
MSKATAQAASFLLLSLLGAAAVARGADPPADTAQIRRGEYLAIAADCVACHTAPGGKPFAGGLPLQIPMLGTIYSSNITPDPNTGIGKWRYEDFERAVRQGVSDDGENLYPAMPYPSYAKINDADMRDLYAYFRYGVAAVESDPPPSTIRWPLNMRWPLKLWNLAFLKSGPYIPKGVKTPTWNRGAYLVQGLAHCGTCHTPRGFAMQEKAMDERGQGYLAGSTLAGWSAYNITSDPASGIGSWKPEQIVQYLRTGSVPGVGQAAGPMGEAVQHSFSRMTETDVRAIAEYLRTVPAVGTGAERARHDWGKPATDVTALRGKPIETTIDAARLYLGNCATCHQADGRGTPDGYYPPLLHNSTVGARDTRNLVQVMLNGIERKAGDRHIGMPAFGRQLSDAQLAALANYVTKQFGDPATPALTAEAIAKRRLPQ

SEQ ID NO: 13 - protein, 427 aa, Ralstonia pickettii
MKAIASFSLLLLAGPLANAWAKDTPADTAQIKRGEYLAIAADCAACHTAPGGKPFAGGLPMQIPMLGTIYSSNITPDEKTGIGKWTYEEFERAVRKGVDDDGNNLYPAMPYPSYAKINDADMRDLYAYFRNGVTAVENRRPRSTIRWPLNMRWPLKLWNLLFLKSEPYTPKSDKSPTWNRGAYLTQGLAHCGTCHTPRGFAMQEKALDERGSGYLAGSTLSGWTAFNITSDPTSGIGAWKPEQLVQYLRTGSVPGVAQAAGPMGEAVQHSFSKMTMQDVQAIAEYLRTVPAVSNNLERARQDWGKPATDVTMLRGKPIETTIDAARLYLGNCASCHQADGRGTPDGYYPPLLHNSTVGTRDTTNLVQVILFGIERKAGDKHIGMPAFARQLSDEQLAALTNYVTRQFGDPATPEVTAEAIAKRRSAK

SEQ ID NO: 14 - DNA, 31 bp, Artificial Sequence
  primer
acgtagccatggcacacaacgacaaccactc

SEQ ID NO: 15 - DNA, 27 bp, Artificial Sequence
  primer
atcggccgcgcgcgcgaagcccggcaa

SEQ ID NO: 16 - DNA, 48 bp, Artificial Sequence
  primer
ttgccgggcttcgcgcgcgcggccgatctgcgcggtgtcgcgctcgcg

SEQ ID NO: 17 - DNA, 48 bp, Artificial Sequence
  primer
ttgccgggcttcgcgcgcgcggccgattatctcggcaactgcgcgacg

SEQ ID NO: 18 - DNA, 42 bp, Artificial Sequence
  primer
gtggtgctcgagtgcggccgcgcgcagcttcgcgacgtcctg

SEQ ID NO: 19 - DNA, 48 bp, Artificial Sequence
  primer
gtacgtaagctttcagtggtggtggtggtggtgctcgagtgcggccgc